European Patent Application EP 4 273 242 A1, published November 8, 2023. Title: CRISPR-BASED MODIFICATION OF HUMAN HBD GENE. Applicant: ETH transfer. The sequence listing filed with the application follows.

SEQUENCE LISTING (91 sequences)

SEQ ID NO: 1 - RNA, 20 nt, Artificial Sequence
  DNA targeting segment 1
aacugcugaaagagaugcgg

SEQ ID NO: 2 - RNA, 20 nt, Artificial Sequence
  DNA targeting segment 2
acugcugaaagagaugcggu

SEQ ID NO: 3 - RNA, 20 nt, Artificial Sequence
  DNA targeting segment 3
cugcugaaagagaugcggug

SEQ ID NO: 4 - RNA, 20 nt, Artificial Sequence
  DNA targeting segment 4
ugcgguggggagauauguag

SEQ ID NO: 5 - RNA, 20 nt, Artificial Sequence
  DNA targeting segment 5
ggagauauguagaggagaac

SEQ ID NO: 6 - RNA, 20 nt, Artificial Sequence
  DNA targeting segment 6
gagauauguagaggagaaca

SEQ ID NO: 7 - RNA, 20 nt, Artificial Sequence
  DNA targeting segment 7
augacagaacagccaaucuc

SEQ ID NO: 8 - RNA, 20 nt, Artificial Sequence
  DNA targeting segment 8
ugacagaacagccaaucuca

SEQ ID NO: 9 - RNA, 20 nt, Artificial Sequence
  DNA targeting segment 9
cccuuaacuugcccugagau

SEQ ID NO: 10 - RNA, 20 nt, Artificial Sequence
  DNA targeting segment 10
gccaaucucagggcaaguua

SEQ ID NO: 11 - RNA, 20 nt, Artificial Sequence
  DNA targeting segment 11
ccaaucucagggcaaguuaa

SEQ ID NO: 12 - RNA, 20 nt, Artificial Sequence
  DNA targeting segment 12
agggcaaguuaagggaauag

SEQ ID NO: 13 - RNA, 20 nt, Artificial Sequence
  DNA targeting segment 13
uuaagggaauaguggaauga

SEQ ID NO: 14 - RNA, 20 nt, Artificial Sequence
  DNA targeting segment 14
agguugguuuaagauaagca

SEQ ID NO: 15 - RNA, 20 nt, Artificial Sequence
  DNA targeting segment 15
cagguugguuuaagauaagc

SEQ ID NO: 16 - RNA, 20 nt, Artificial Sequence
  DNA targeting segment 16
cccugcuccagugagcaggu

SEQ ID NO: 17 - RNA, 20 nt, Artificial Sequence
  DNA targeting segment 17
ucuuaaaccaaccugcucac

SEQ ID NO: 18 - RNA, 20 nt, Artificial Sequence
  DNA targeting segment 18
uccucccugcuccagugagc

SEQ ID NO: 19 - RNA, 20 nt, Artificial Sequence
  DNA targeting segment 19
accaaccugcucacuggagc

SEQ ID NO: 20 - RNA, 20 nt, Artificial Sequence
  DNA targeting segment 20
ccaaccugcucacuggagca

SEQ ID NO: 21 - RNA, 20 nt, Artificial Sequence
  DNA targeting segment 21
accugcucacuggagcaggg

SEQ ID NO: 22 - RNA, 20 nt, Artificial Sequence
  DNA targeting segment 22
cucacuggagcagggaggac

SEQ ID NO: 23 - RNA, 20 nt, Artificial Sequence
  DNA targeting segment 23
cucugcccugccuuuuaugc

SEQ ID NO: 24 - RNA, 20 nt, Artificial Sequence
  DNA targeting segment 24
gaggacaggaccagcauaaa

SEQ ID NO: 25 - RNA, 20 nt, Artificial Sequence
  DNA targeting segment 25
acaggaccagcauaaaaggc

SEQ ID NO: 26 - RNA, 20 nt, Artificial Sequence
  DNA targeting segment 26
caggaccagcauaaaaggca

SEQ ID NO: 27 - RNA, 20 nt, Artificial Sequence
  DNA targeting segment 27
ugcaccauggugucuguuug

SEQ ID NO: 28 - RNA, 20 nt, Artificial Sequence
  DNA targeting segment 28
gcaaccucaaacagacacca

SEQ ID NO: 29 - RNA, 20 nt, Artificial Sequence
  DNA targeting segment 29
cucaggagucagaugcacca

SEQ ID NO: 30 - RNA, 20 nt, Artificial Sequence
  DNA targeting segment 30
cauggugcaucugacuccug

SEQ ID NO: 31 - RNA, 20 nt, Artificial Sequence
  DNA targeting segment 31
uugacagcagucuucuccuc

SEQ ID NO: 32 - RNA, 20 nt, Artificial Sequence
  DNA targeting segment 32
agacugcugucaaugcccug

SEQ ID NO: 33 - RNA, 20 nt, Artificial Sequence
  DNA targeting segment 33
gacugcugucaaugcccugu

SEQ ID NO: 34 - RNA, 20 nt, Artificial Sequence
  DNA targeting segment 34ACUGCUGUCAAUGCCCUGUG
acugcugucaaugcccugug

SEQ ID NO: 35 - RNA, 20 nt, Artificial Sequence
  DNA targeting segment 35
cacguucacuuugccccaca

SEQ ID NO: 36 - RNA, 20 nt, Artificial Sequence
  DNA targeting segment 36
ccacguucacuuugccccac

SEQ ID NO: 37 - RNA, 20 nt, Artificial Sequence
  DNA targeting segment 37
ccuguggggcaaagugaacg

SEQ ID NO: 38 - RNA, 20 nt, Artificial Sequence
  DNA targeting segment 38
aaagugaacguggaugcagu

SEQ ID NO: 39 - RNA, 20 nt, Artificial Sequence
  DNA targeting segment 39
gugaacguggaugcaguugg

SEQ ID NO: 40 - RNA, 20 nt, Artificial Sequence
  DNA targeting segment 40
cguggaugcaguugguggug

SEQ ID NO: 41 - RNA, 20 nt, Artificial Sequence
  DNA targeting segment 41
ugcaguugguggugaggccc

SEQ ID NO: 42 - RNA, 20 nt, Artificial Sequence
  DNA targeting segment 42
gcaguugguggugaggcccu

SEQ ID NO: 43 - RNA, 20 nt, Artificial Sequence
  DNA targeting segment 43
uugguggugaggcccugggc

SEQ ID NO: 44 - RNA, 82 nt, Artificial Sequence
  Exemplary scaffold region
guuuuagagcuagaaatagcaaguuaaaauaaggcuaguccguuaucaacuugaaaaaguggcaccgagucggugcuuuuuu

SEQ ID NO: 45 - RNA, 102 nt, Artificial Sequence
  exemplary gRNA
cagguugguuuaagauaagcguuuuagagcuagaaatagcaaguuaaaauaaggcuaguccguuaucaacuugaaaaaguggcaccgagucggugcuuuuuu

SEQ ID NO: 46 - RNA, 102 nt, Artificial Sequence
  Exemplary gRNA
cucugcccugccuuuuaugcguuuuagagcuagaaatagcaaguuaaaauaaggcuaguccguuaucaacuugaaaaaguggcaccgagucggugcuuuuuu

SEQ ID NO: 47 - RNA, 102 nt, Artificial Sequence
  Exemplary gRNA
caggaccagcauaaaaggcaguuuuagagcuagaaatagcaaguuaaaauaaggcuaguccguuaucaacuugaaaaaguggcaccgagucggugcuuuuuu

SEQ ID NO: 48 - RNA, 102 nt, Artificial Sequence
  Exemplary gRNA
acaggaccagcauaaaaggcguuuuagagcuagaaatagcaaguuaaaauaaggcuaguccguuaucaacuugaaaaaguggcaccgagucggugcuuuuuu

SEQ ID NO: 49 - RNA, 102 nt, Artificial Sequence
  Exemplary gRNA
agguugguuuaagauaagcaguuuuagagcuagaaatagcaaguuaaaauaaggcuaguccguuaucaacuugaaaaaguggcaccgagucggugcuuuuuu

SEQ ID NO: 50 - DNA, 199 bp, Artificial Sequence
  Exemplary first homology arm sequence
attagcctaaaacacttctgcaaaaatgaaactaggaggatatttttagaaacaactgctgaaagagatgcggtggggagatatgtagaggagaacagggtttctgagtcaagacacacatgacagaacagccaatctcagggcaagttaagggaatagtggaatgaaggttcatttttcattctcacaaactaatgaa

SEQ ID NO: 51 - DNA, 200 bp, Artificial Sequence
  Exemplary second homology arm sequence
gcagggcagagtcgactgttgcttacactttcttctgacataacagtgttcactagcaacctcaaacagacaccatggtgcatctgactcctgaggagaagactgctgtcaatgccctgtggggcaaagtgaacgtggatgcagttggtggtgaggccctgggcaggttggtatcaaggttataagagaggctcaaggag

SEQ ID NO: 52-54 - skipped (3 entries)

SEQ ID NO: 55 - DNA, 194 bp, Artificial Sequence
  Exemplary DNA donor template
ggaatagtggaatgaaggttcatttttcattctcacaaactaatgaaaccctgcttatcttaaaccaacctgctcaccacaccctggagcagggagggcaggagccagggctgggcataaaaggcagggcagagtcgactgttgcttacactttcttctgacataacagtgttcactagcaacctcaaacagac

SEQ ID NO: 56 - protein, 1368 aa, Artificial Sequence [sequence omitted]

SEQ ID NO: 57 - DNA, 4104 bp, Artificial Sequence
  SpCas9 DNA
atggacaagaagtacagcatcggcctggacatcggcaccaactctgtgggctgggccgtgatcaccgacgagtacaaggtgcccagcaagaaattcaaggtgctgggcaacaccgaccggcacagcatcaagaagaacctgatcggagccctgctgttcgacagcggcgaaacagccgaggccacccggctgaagagaaccgccagaagaagatacaccagacggaagaaccggatctgctatctgcaagagatcttcagcaacgagatggccaaggtggacgacagcttcttccacagactggaagagtccttcctggtggaagaggataagaagcacgagcggcaccccatcttcggcaacatcgtggacgaggtggcctaccacgagaagtaccccaccatctaccacctgagaaagaaactggtggacagcaccgacaaggccgacctgcggctgatctatctggccctggcccacatgatcaagttccggggccacttcctgatcgagggcgacctgaaccccgacaacagcgacgtggacaagctgttcatccagctggtgcagacctacaaccagctgttcgaggaaaaccccatcaacgccagcggcgtggacgccaaggccatcctgtctgccagactgagcaagagcagacggctggaaaatctgatcgcccagctgcccggcgagaagaagaatggcctgttcggaaacctgattgccctgagcctgggcctgacccccaacttcaagagcaacttcgacctggccgaggatgccaaactgcagctgagcaaggacacctacgacgacgacctggacaacctgctggcccagatcggcgaccagtacgccgacctgtttctggccgccaagaacctgtccgacgccatcctgctgagcgacatcctgagagtgaacaccgagatcaccaaggcccccctgagcgcctctatgatcaagagatacgacgagcaccaccaggacctgaccctgctgaaagctctcgtgcggcagcagctgcctgagaagtacaaagagattttcttcgaccagagcaagaacggctacgccggctacattgacggcggagccagccaggaagagttctacaagttcatcaagcccatcctggaaaagatggacggcaccgaggaactgctcgtgaagctgaacagagaggacctgctgcggaagcagcggaccttcgacaacggcagcatcccccaccagatccacctgggagagctgcacgccattctgcggcggcaggaagatttttacccattcctgaaggacaaccgggaaaagatcgagaagatcctgaccttccgcatcccctactacgtgggccctctggccaggggaaacagcagattcgcctggatgaccagaaagagcgaggaaaccatcaccccctggaacttcgaggaagtggtggacaagggcgcttccgcccagagcttcatcgagcggatgaccaacttcgataagaacctgcccaacgagaaggtgctgcccaagcacagcctgctgtacgagtacttcaccgtgtataacgagctgaccaaagtgaaatacgtgaccgagggaatgagaaagcccgccttcctgagcggcgagcagaaaaaggccatcgtggacctgctgttcaagaccaaccggaaagtgaccgtgaagcagctgaaagaggactacttcaagaaaatcgagtgcttcgactccgtggaaatctccggcgtggaagatcggttcaacgcctccctgggcacataccacgatctgctgaaaattatcaaggacaaggacttcctggacaatgaggaaaacgaggacattctggaagatatcgtgctgaccctgacactgtttgaggacagagagatgatcgaggaacggctgaaaacctatgcccacctgttcgacgacaaagtgatgaagcagctgaagcggcggagatacaccggctggggcaggctgagccggaagctgatcaacggcatccgggacaagcagtccggcaagacaatcctggatttcctgaagtccgacggcttcgccaacagaaacttcatgcagctgatccacgacgacagcctgacctttaaagaggacatccagaaagcccaggtgtccggccagggcgatagcctgcacgagcacattgccaatctggccggcagccccgccattaagaagggcatcctgcagacagtgaaggtggtggacgagctcgtgaaagtgatgggccggcacaagcccgagaacatcgtgatcgaaatggccagagagaaccagaccacccagaagggacagaagaacagccgcgagagaatgaagcggatcgaagagggcatcaaagagctgggcagccagatcctgaaagaacaccccgtggaaaacacccagctgcagaacgagaagctgtacctgtactacctgcagaatgggcgggatatgtacgtggaccaggaactggacatcaaccggctgtccgactacgatgtggaccatatcgtgcctcagagctttctgaaggacgactccatcgacaacaaggtgctgaccagaagcgacaagaaccggggcaagagcgacaacgtgccctccgaagaggtcgtgaagaagatgaagaactactggcggcagctgctgaacgccaagctgattacccagagaaagttcgacaatctgaccaaggccgagagaggcggcctgagcgaactggataaggccggcttcatcaagagacagctggtggaaacccggcagatcacaaagcacgtggcacagatcctggactcccggatgaacactaagtacgacgagaatgacaagctgatccgggaagtgaaagtgatcaccctgaagtccaagctggtgtccgatttccggaaggatttccagttttacaaagtgcgcgagatcaacaactaccaccacgcccacgacgcctacctgaacgccgtcgtgggaaccgccctgatcaaaaagtaccctaagctggaaagcgagttcgtgtacggcgactacaaggtgtacgacgtgcggaagatgatcgccaagagcgagcaggaaatcggcaaggctaccgccaagtacttcttctacagcaacatcatgaactttttcaagaccgagattaccctggccaacggcgagatccggaagcggcctctgatcgagacaaacggcgaaaccggggagatcgtgtgggataagggccgggattttgccaccgtgcggaaagtgctgagcatgccccaagtgaatatcgtgaaaaagaccgaggtgcagacaggcggcttcagcaaagagtctatcctgcccaagaggaacagcgataagctgatcgccagaaagaaggactgggaccctaagaagtacggcggcttcgacagccccaccgtggcctattctgtgctggtggtggccaaagtggaaaagggcaagtccaagaaactgaagagtgtgaaagagctgctggggatcaccatcatggaaagaagcagcttcgagaagaatcccatcgactttctggaagccaagggctacaaagaagtgaaaaaggacctgatcatcaagctgcctaagtactccctgttcgagctggaaaacggccggaagagaatgctggcctctgccggcgaactgcagaagggaaacgaactggccctgccctccaaatatgtgaacttcctgtacctggccagccactatgagaagctgaagggctcccccgaggataatgagcagaaacagctgtttgtggaacagcacaagcactacctggacgagatcatcgagcagatcagcgagttctccaagagagtgatcctggccgacgctaatctggacaaagtgctgtccgcctacaacaagcaccgggataagcccatcagagagcaggccgagaatatcatccacctgtttaccctgaccaatctgggagcccctgccgccttcaagtactttgacaccaccatcgaccggaagaggtacaccagcaccaaagaggtgctggacgccaccctgatccaccagagcatcaccggcctgtacgagacacggatcgacctgtctcagctgggaggcgac

SEQ ID NO: 58 - protein, 1367 aa, Artificial Sequence
  HiFi Cas9 AA
DKKYSIGLDIGTNSVGWAVITDEYKVPSKKFKVLGNTDRHSIKKNLIGALLFDSGETAEATRLKRTARRRYTRRKNRICYLQEIFSNEMAKVDDSFFHRLEESFLVEEDKKHERHPIFGNIVDEVAYHEKYPTIYHLRKKLVDSTDKADLRLIYLALAHMIKFRGHFLIEGDLNPDNSDVDKLFIQLVQTYNQLFEENPINASGVDAKAILSARLSKSRRLENLIAQLPGEKKNGLFGNLIALSLGLTPNFKSNFDLAEDAKLQLSKDTYDDDLDNLLAQIGDQYADLFLAAKNLSDAILLSDILRVNTEITKAPLSASMIKRYDEHHQDLTLLKALVRQQLPEKYKEIFFDQSKNGYAGYIDGGASQEEFYKFIKPILEKMDGTEELLVKLNREDLLRKQRTFDNGSIPHQIHLGELHAILRRQEDFYPFLKDNREKIEKILTFRIPYYVGPLARGNSRFAWMTRKSEETITPWNFEEVVDKGASAQSFIERMTNFDKNLPNEKVLPKHSLLYEYFTVYNELTKVKYVTEGMRKPAFLSGEQKKAIVDLLFKTNRKVTVKQLKEDYFKKIECFDSVEISGVEDRFNASLGTYHDLLKIIKDKDFLDNEENEDILEDIVLTLTLFEDREMIEERLKTYAHLFDDKVMKQLKRRRYTGWGRLSRKLINGIRDKQSGKTILDFLKSDGFANANFMQLIHDDSLTFKEDIQKAQVSGQGDSLHEHIANLAGSPAIKKGILQTVKVVDELVKVMGRHKPENIVIEMARENQTTQKGQKNSRERMKRIEEGIKELGSQILKEHPVENTQLQNEKLYLYYLQNGRDMYVDQELDINRLSDYDVDHIVPQSFLKDDSIDNKVLTRSDKNRGKSDNVPSEEVVKKMKNYWRQLLNAKLITQRKFDNLTKAERGGLSELDKAGFIKRQLVETRQITKHVAQILDSRMNTKYDENDKLIREVKVITLKSKLVSDFRKDFQFYKVREINNYHHAHDAYLNAVVGTALIKKYPKLESEFVYGDYKVYDVRKMIAKSEQEIGKATAKYFFYSNIMNFFKTEITLANGEIRKRPLIETNGETGEIVWDKGRDFATVRKVLSMPQVNIVKKTEVQTGGFSKESILPKRNSDKLIARKKDWDPKKYGGFDSPTVAYSVLVVAKVEKGKSKKLKSVKELLGITIMERSSFEKNPIDFLEAKGYKEVKKDLIIKLPKYSLFELENGRKRMLASAGELQKGNELALPSKYVNFLYLASHYEKLKGSPEDNEQKQLFVEQHKHYLDEIIEQISEFSKRVILADANLDKVLSAYNKHRDKPIREQAENIIHLFTLTNLGAPAAFKYFDTTIDRKRYTSTKEVLDATLIHQSITGLYETRIDLSQLGGD

SEQ ID NO: 59 - DNA, 4101 bp, Artificial Sequence
  HiFi Cas9 DNA
gacaagaagtacagcatcggcctggacatcggcaccaactctgtgggctgggccgtgatcaccgacgagtacaaggtgcccagcaagaaattcaaggtgctgggcaacaccgaccggcacagcatcaagaagaacctgatcggagcgctgctgttcgacagcggcgaaacagccgaggccacccggcttaagagaaccgccagaagaagatacaccagacggaagaaccggatctgctatctgcaagagatcttcagcaacgagatggccaaggtggacgacagcttcttccacagactggaagagtccttcctggtggaagaggataagaagcacgagcggcaccccatcttcggcaacatcgtggacgaggtggcctaccacgagaagtaccccaccatctaccacctgagaaagaaactggtggacagcaccgacaaggccgacctgcggctgatctatctggccctggcccacatgatcaagttccggggccacttcctgatcgagggcgacctgaaccccgacaacagcgacgtggacaagctgttcatccagctggtgcagacctacaaccagctgttcgaggaaaaccccatcaacgccagcggcgtggacgccaaggccatcctgtctgccagactgagcaagagcagacggctggaaaatctgatcgcccagctgcccggcgagaagaagaatggcctgttcggaaacctgattgccctgagcctgggcctgacccccaacttcaagagcaacttcgacctggccgaggatgccaaactgcagctgagcaaggacacctacgacgacgacctggacaacctgctggcccagatcggcgaccagtacgccgacctgtttctggccgccaagaacctgtccgacgccatcctgctgagcgacatcctgagagtgaacaccgagatcaccaaggcccccctgagcgcctctatgatcaagagatacgacgagcaccaccaggacctgaccctgctgaaagctctcgtgcggcagcagctgcctgagaagtacaaagagattttcttcgaccagagcaagaacggctacgccggctacattgacggcggagccagccaggaagagttctacaagttcatcaagcccatcctggaaaagatggacggcaccgaggaactgctcgtgaagctgaacagagaggacctcctgaggaagcagcggaccttcgacaacggcagcatcccccaccagatccacctgggagagctgcacgccattctgcggcggcaggaagatttttacccattcctgaaggacaaccgggaaaagatcgagaagatcctgaccttccgcatcccctactacgtgggccctctggccaggggaaacagcagattcgcctggatgaccagaaagagcgaggaaaccatcaccccctggaacttcgaggaagtggtggacaagggcgcttccgcccagagcttcatcgagcggatgaccaacttcgataagaacctgcccaacgagaaggtgctgcccaagcacagcctgctgtacgagtacttcaccgtgtataacgagctgaccaaagtgaaatacgtgaccgagggaatgagaaagcccgccttcctgagcggcgagcagaaaaaggccatcgtggacctgctgttcaagaccaaccggaaagtgaccgtgaagcagctgaaagaggactacttcaagaaaatcgagtgcttcgactccgtggaaatctccggcgtggaagatcggttcaacgcctccctgggcacataccacgatctgctgaaaattatcaaggacaaggacttcctggacaatgaggaaaacgaggacattctggaagatatcgtgctgaccctgacactgtttgaggacagagagatgatcgaggaacggctgaaaacctatgcccacctgttcgacgacaaagtgatgaagcagctgaagcggcggagatacaccggctggggcaggctgagccggaagctgatcaacggcatccgggacaagcagtccggcaagacaatcctggatttcctgaagtccgacggcttcgccaacgccaacttcatgcaattgatccacgacgacagcctgacctttaaagaggacatccagaaagcccaggtgtccggccagggcgatagtctacacgagcacattgccaatctggccggcagccccgccattaagaagggcatcctgcagacagtgaaggtggtggacgagctcgtgaaagtgatgggccggcacaagcccgagaacatcgtgatcgaaatggccagagagaaccagaccacccagaagggacagaagaacagccgcgagagaatgaagcggatcgaagagggcatcaaagagctgggcagccagatcctgaaagaacaccccgtggaaaacacccagctgcagaacgagaagctgtacctgtactacctgcagaatgggcgggatatgtacgtggaccaggaactggacatcaaccggctgtccgactacgatgtggaccatatcgtgcctcagagctttctgaaggacgactccatcgacaacaaggtgctgaccagaagcgacaagaaccggggcaagagcgacaacgtgccctccgaagaggtcgtgaagaagatgaagaactactggcggcagctgctgaacgccaagcttattacccagagaaagttcgacaatctgaccaaggccgagagaggcggcctgagcgaactggataaggccggcttcatcaagagacagctggtggaaacccggcagatcacaaagcacgtggcacagatcctggactcccggatgaacactaagtacgacgagaatgacaagctgatccgggaagtgaaagtgatcaccctgaagtccaagctggtgtccgatttccggaaggatttccagttttacaaagtgcgcgagatcaacaactaccaccacgcccacgacgcctacctgaacgccgtcgtgggaaccgccctgatcaaaaagtaccctaagctcgagagcgagttcgtgtacggcgactacaaggtgtacgacgtgcggaagatgatcgccaagagcgagcaggaaatcggcaaggctaccgccaagtacttcttctacagcaacatcatgaactttttcaagaccgagattaccctggccaacggcgagatccggaagcggcctctgatcgagacaaacggcgaaaccggggagatcgtgtgggataagggccgggattttgccaccgtgcggaaagtgctgagcatgccccaagtgaatatcgtgaaaaagaccgaggtgcagacaggcggcttcagcaaagagtctatcctgcccaagaggaacagcgataagctgatcgccagaaagaaggactgggaccctaagaagtacggcggcttcgacagccccaccgtggcctattctgtgctggtggtggccaaagtggaaaagggcaagtccaagaaactgaagagtgtgaaagagctgctggggatcaccatcatggaaagaagcagcttcgagaagaatcccatcgactttctggaagccaagggctacaaagaagtgaaaaaggacctgatcatcaagctgcctaagtactccctgttcgagctggaaaacggccggaagagaatgctggcctctgccggcgaactgcagaagggaaacgaactggccctgccctccaaatatgtgaacttcctgtacctggccagccactatgagaagctgaagggctcccccgaggataatgagcagaaacagctgtttgtggaacagcacaagcactacctggacgagatcatcgagcagatcagcgagttctccaagagagtgatcctggccgacgctaatctggacaaagtgctgtccgcctacaacaagcaccgggataagcccatcagagagcaggccgagaatatcatccacctgtttaccctgaccaatctgggagcccctgccgccttcaagtactttgacaccaccatcgaccggaagaggtacaccagcaccaaagaggtgctggacgccaccctgatccaccagagcatcaccggcctgtacgagacacggatcgacctgtctcagctgggaggcgac

SEQ ID NO: 60 - protein, 1368 aa, Artificial Sequence
  SpRY Cas9 AA
MDKKYSIGLDIGTNSVGWAVITDEYKVPSKKFKVLGNTDRHSIKKNLIGALLFDSGETAERTRLKRTARRRYTRRKNRICYLQEIFSNEMAKVDDSFFHRLEESFLVEEDKKHERHPIFGNIVDEVAYHEKYPTIYHLRKKLVDSTDKADLRLIYLALAHMIKFRGHFLIEGDLNPDNSDVDKLFIQLVQTYNQLFEENPINASGVDAKAILSARLSKSRRLENLIAQLPGEKKNGLFGNLIALSLGLTPNFKSNFDLAEDAKLQLSKDTYDDDLDNLLAQIGDQYADLFLAAKNLSDAILLSDILRVNTEITKAPLSASMIKRYDEHHQDLTLLKALVRQQLPEKYKEIFFDQSKNGYAGYIDGGASQEEFYKFIKPILEKMDGTEELLVKLNREDLLRKQRTFDNGSIPHQIHLGELHAILRRQEDFYPFLKDNREKIEKILTFRIPYYVGPLARGNSRFAWMTRKSEETITPWNFEEVVDKGASAQSFIERMTNFDKNLPNEKVLPKHSLLYEYFTVYNELTKVKYVTEGMRKPAFLSGEQKKAIVDLLFKTNRKVTVKQLKEDYFKKIECFDSVEISGVEDRFNASLGTYHDLLKIIKDKDFLDNEENEDILEDIVLTLTLFEDREMIEERLKTYAHLFDDKVMKQLKRRRYTGWGRLSRKLINGIRDKQSGKTILDFLKSDGFANRNFMQLIHDDSLTFKEDIQKAQVSGQGDSLHEHIANLAGSPAIKKGILQTVKVVDELVKVMGRHKPENIVIEMARENQTTQKGQKNSRERMKRIEEGIKELGSQILKEHPVENTQLQNEKLYLYYLQNGRDMYVDQELDINRLSDYDVDHIVPQSFLKDDSIDNKVLTRSDKNRGKSDNVPSEEVVKKMKNYWRQLLNAKLITQRKFDNLTKAERGGLSELDKAGFIKRQLVETRQITKHVAQILDSRMNTKYDENDKLIREVKVITLKSKLVSDFRKDFQFYKVREINNYHHAHDAYLNAVVGTALIKKYPKLESEFVYGDYKVYDVRKMIAKSEQEIGKATAKYFFYSNIMNFFKTEITLANGEIRKRPLIETNGETGEIVWDKGRDFATVRKVLSMPQVNIVKKTEVQTGGFSKESIRPKRNSDKLIARKKDWDPKKYGGFLWPTVAYSVLVVAKVEKGKSKKLKSVKELLGITIMERSSFEKNPIDFLEAKGYKEVKKDLIIKLPKYSLFELENGRKRMLASAKQLQKGNELALPSKYVNFLYLASHYEKLKGSPEDNEQKQLFVEQHKHYLDEIIEQISEFSKRVILADANLDKVLSAYNKHRDKPIREQAENIIHLFTLTRLGAPRAFKYFDTTIDPKQYRSTKEVLDATLIHQSITGLYETRIDLSQLGGD

SEQ ID NO: 61 - DNA, 4104 bp, Artificial Sequence
  SpRY Cas9 DNA
atggacaagaagtacagcatcggcctggacatcggcaccaactctgtgggctgggccgtgatcaccgacgagtacaaggtgcccagcaagaaattcaaggtgctgggcaacaccgaccggcacagcatcaagaagaacctgatcggagccctgctgttcgacagcggcgaaacagccgagagaacccggctgaagagaaccgccagaagaagatacaccagacggaagaaccggatctgctatctgcaagagatcttcagcaacgagatggccaaggtggacgacagcttcttccacagactggaagagtccttcctggtggaagaggataagaagcacgagcggcaccccatcttcggcaacatcgtggacgaggtggcctaccacgagaagtaccccaccatctaccacctgagaaagaaactggtggacagcaccgacaaggccgacctgcggctgatctatctggccctggcccacatgatcaagttccggggccacttcctgatcgagggcgacctgaaccccgacaacagcgacgtggacaagctgttcatccagctggtgcagacctacaaccagctgttcgaggaaaaccccatcaacgccagcggcgtggacgccaaggccatcctgtctgccagactgagcaagagcagacggctggaaaatctgatcgcccagctgcccggcgagaagaagaatggcctgttcggaaacctgattgccctgagcctgggcctgacccccaacttcaagagcaacttcgacctggccgaggatgccaaactgcagctgagcaaggacacctacgacgacgacctggacaacctgctggcccagatcggcgaccagtacgccgacctgtttctggccgccaagaacctgtccgacgccatcctgctgagcgacatcctgagagtgaacaccgagatcaccaaggcccccctgagcgcctctatgatcaagagatacgacgagcaccaccaggacctgaccctgctgaaagctctcgtgcggcagcagctgcctgagaagtacaaagagattttcttcgaccagagcaagaacggctacgccggctacattgacggcggagccagccaggaagagttctacaagttcatcaagcccatcctggaaaagatggacggcaccgaggaactgctcgtgaagctgaacagagaggacctgctgcggaagcagcggaccttcgacaacggcagcatcccccaccagatccacctgggagagctgcacgccattctgcggcggcaggaagatttttacccattcctgaaggacaaccgggaaaagatcgagaagatcctgaccttccgcatcccctactacgtgggccctctggccaggggaaacagcagattcgcctggatgaccagaaagagcgaggaaaccatcaccccctggaacttcgaggaagtggtggacaagggcgcttccgcccagagcttcatcgagcggatgaccaacttcgataagaacctgcccaacgagaaggtgctgcccaagcacagcctgctgtacgagtacttcaccgtgtataacgagctgaccaaagtgaaatacgtgaccgagggaatgagaaagcccgccttcctgagcggcgagcagaaaaaggccatcgtggacctgctgttcaagaccaaccggaaagtgaccgtgaagcagctgaaagaggactacttcaagaaaatcgagtgcttcgactccgtggaaatctccggcgtggaagatcggttcaacgcctccctgggcacataccacgatctgctgaaaattatcaaggacaaggacttcctggacaatgaggaaaacgaggacattctggaagatatcgtgctgaccctgacactgtttgaggacagagagatgatcgaggaacggctgaaaacctatgcccacctgttcgacgacaaagtgatgaagcagctgaagcggcggagatacaccggctggggcaggctgagccggaagctgatcaacggcatccgggacaagcagtccggcaagacaatcctggatttcctgaagtccgacggcttcgccaacagaaacttcatgcagctgatccacgacgacagcctgacctttaaagaggacatccagaaagcccaggtgtccggccagggcgatagcctgcacgagcacattgccaatctggccggcagccccgccattaagaagggcatcctgcagacagtgaaggtggtggacgagctcgtgaaagtgatgggccggcacaagcccgagaacatcgtgatcgaaatggccagagagaaccagaccacccagaagggacagaagaacagccgcgagagaatgaagcggatcgaagagggcatcaaagagctgggcagccagatcctgaaagaacaccccgtggaaaacacccagctgcagaacgagaagctgtacctgtactacctgcagaatgggcgggatatgtacgtggaccaggaactggacatcaaccggctgtccgactacgatgtggaccatatcgtgcctcagagctttctgaaggacgactccatcgacaacaaggtgctgaccagaagcgacaagaaccggggcaagagcgacaacgtgccctccgaagaggtcgtgaagaagatgaagaactactggcggcagctgctgaacgccaagctgattacccagagaaagttcgacaatctgaccaaggccgagagaggcggcctgagcgaactggataaggccggcttcatcaagagacagctggtggaaacccggcagatcacaaagcacgtggcacagatcctggactcccggatgaacactaagtacgacgagaatgacaagctgatccgggaagtgaaagtgatcaccctgaagtccaagctggtgtccgatttccggaaggatttccagttttacaaagtgcgcgagatcaacaactaccaccacgcccacgacgcctacctgaacgccgtcgtgggaaccgccctgatcaaaaagtaccctaagctggaaagcgagttcgtgtacggcgactacaaggtgtacgacgtgcggaagatgatcgccaagagcgagcaggaaatcggcaaggctaccgccaagtacttcttctacagcaacatcatgaactttttcaagaccgagattaccctggccaacggcgagatccggaagcggcctctgatcgagacaaacggcgaaaccggggagatcgtgtgggataagggccgggattttgccaccgtgcggaaagtgctgagcatgccccaagtgaatatcgtgaaaaagaccgaggtgcagacaggcggcttcagcaaagagtctatcagacccaagaggaacagcgataagctgatcgccagaaagaaggactgggaccctaagaagtacggcggcttcctgtggcccaccgtggcctattctgtgctggtggtggccaaagtggaaaagggcaagtccaagaaactgaagagtgtgaaagagctgctggggatcaccatcatggaaagaagcagcttcgagaagaatcccatcgactttctggaagccaagggctacaaagaagtgaaaaaggacctgatcatcaagctgcctaagtactccctgttcgagctggaaaacggccggaagagaatgctggcctctgccaagcagctgcagaagggaaacgaactggccctgccctccaaatatgtgaacttcctgtacctggccagccactatgagaagctgaagggctcccccgaggataatgagcagaaacagctgtttgtggaacagcacaagcactacctggacgagatcatcgagcagatcagcgagttctccaagagagtgatcctggccgacgctaatctggacaaagtgctgtccgcctacaacaagcaccgggataagcccatcagagagcaggccgagaatatcatccacctgtttaccctgaccagactgggagcccctagagccttcaagtactttgacaccaccatcgaccccaagcagtacagaagcaccaaagaggtgctggacgccaccctgatccaccagagcatcaccggcctgtacgagacacggatcgacctgtctcagctgggaggcgac

SEQ ID NO: 62 - protein, 1306 aa, Artificial Sequence
  Cpf1 AA
MTQFEGFTNLYQVSKTLRFELIPQGKTLKHIQEQGFIEEDKARNDHYKELKPIIDRIYKTYADQCLQLVQLDWENLSAAIDSYRKEKTEETRNALIEEQATYRNAIHDYFIGRTDNLTDAINKRHAEIYKGLFKAELFNGKVLKQLGTVTTTEHENALLRSFDKFTTYFSGFYRNRKNVFSAEDISTAIPHRIVQDNFPKFKENCHIFTRLITAVPSLREHFENVKKAIGIFVSTSIEEVFSFPFYNQLLTQTQIDLYNQLLGGISREAGTEKIKGLNEVLALAIQKNDETAHIIASLPHRFIPLFKQILSDRNTLSFILEEFKSDEEVIQSFCKYKTLLRNENVLETAEALFNELNSIDLTHIFISHKKLETISSALCDHWDTLRNALYERRISELTGKITKSAKEKVQRSLKHEDINLQEIISAAGKELSEAFKQKTSEILSHAHAALDQPLPTTLKKQEEKEILKSQLDSLLGLYHLLDWFAVDESNEVDPEFSARLTGIKLEMEPSLSFYNKARNYATKKPYSVEKFKLNFQMPTLARGWDVNREKNNGAILFVKNGLYYLGIMPKQKGRYKALSFEPTEKTSEGFDKMYYDYFPDAAKMIPKCSTQLKAVTAHFQTHTTPILLSNNFIEPLEITKEIYDLNNPEKEPKKFQTAYAKKTGDQKGYREALCKWIDFTRDFLSKYTKTTSIDLSSLRPSSQYKDLGEYYAELNPLLYHISFQRIAEKEIMDAVETGKLYLFQIYNKDFAKGHHGKPNLHTLYWTGLFSPENLAKTSIKLNGQAELFYRPKSRMKRMAHRLGEKMLNKKLKDQKTPIPDTLYQELYDYVNHRLSHDLSDEARALLPNVITKEVSHEIIKDRRFTSDKFFFHVPITLNYQAANSPSKFNQRVNAYLKEHPETPIIGIDRGERNLIYITVIDSTGKILEQRSLNTIQQFDYQKKLDNREKERVAARQAWSVVGTIKDLKQGYLSQVIHEIVDLMIHYQAVVVLENLNFGFKSKRTGIAEKAVYQQFEKMLIDKLNCLVLKDYPAEKVGGVLNPYQLTDQFTSFAKMGTQSGFLFYVPAPYTSKIDPLTGFVDPFVWKTIKNHESRKHFLEGFDFLHYDVKTGDFILHFKMNRNLSFQRGLPGFMPAWDIVFEKNETQFDAKGTPFIAGKRIVPVIENHRFTGRYRDLYPANELIALLEEKGIVFRDGSNILPKLLENDDSHAIDTMVALIRSVLQMRNSNAATGEDYINSPVRDLNGVCFDSRFQNPEWPMDADANGAYHIALKGQLLLNHLKESKDLKLQNGISNQDWLAYIQELR

SEQ ID NO: 63 - DNA, 3921 bp, Artificial Sequence
  Cpf1 DNA
atgacacagttcgagggctttaccaacctgtatcaggtgagcaagacactgcggtttgagctgatcccacagggcaagaccctgaagcacatccaggagcagggcttcatcgaggaggacaaggcccgcaatgatcactacaaggagctgaagcccatcatcgatcggatctacaagacctatgccgaccagtgcctgcagctggtgcagctggattgggagaacctgagcgccgccatcgactcctatagaaaggagaaaaccgaggagacaaggaacgccctgatcgaggagcaggccacatatcgcaatgccatccacgactacttcatcggccggacagacaacctgaccgatgccatcaataagagacacgccgagatctacaagggcctgttcaaggccgagctgtttaatggcaaggtgctgaagcagctgggcaccgtgaccacaaccgagcacgagaacgccctgctgcggagcttcgacaagtttacaacctacttctccggcttttatagaaacaggaagaacgtgttcagcgccgaggatatcagcacagccatcccacaccgcatcgtgcaggacaacttccccaagtttaaggagaattgtcacatcttcacacgcctgatcaccgccgtgcccagcctgcgggagcactttgagaacgtgaagaaggccatcggcatcttcgtgagcacctccatcgaggaggtgttttccttccctttttataaccagctgctgacacagacccagatcgacctgtataaccagctgctgggaggaatctctcgggaggcaggcaccgagaagatcaagggcctgaacgaggtgctggccctggccatccagaagaatgatgagacagcccacatcatcgcctccctgccacacagattcatccccctgtttaagcagatcctgtccgataggaacaccctgtctttcatcctggaggagtttaagagcgacgaggaagtgatccagtccttctgcaagtacaagacactgctgagaaacgagaacgtgctggagacagccgaggccctgtttaacgagctgaacagcatcgacctgacacacatcttcatcagccacaagaagctggagacaatcagcagcgccctgtgcgaccactgggatacactgaggaatgccctgtatgagcggagaatctccgagctgacaggcaagatcaccaagtctgccaaggagaaggtgcagcgcagcctgaagcacgaggatatcaacctgcaggagatcatctctgccgcaggcaaggagctgagcgaggccttcaagcagaaaaccagcgagatcctgtcccacgcacacgccgccctggatcagccactgcctacaaccctgaagaagcaggaggagaaggagatcctgaagtctcagctggacagcctgctgggcctgtaccacctgctggactggtttgccgtggatgagtccaacgaggtggaccccgagttctctgcccggctgaccggcatcaagctggagatggagccttctctgagcttctacaacaaggccagaaattatgccaccaagaagccctactccgtggagaagttcaagctgaactttcagatgcctacactggccagaggctgggacgtgaatagagagaagaacaatggcgccatcctgtttgtgaagaacggcctgtactatctgggcatcatgccaaagcagaagggcaggtataaggccctgagcttcgagcccacagagaaaaccagcgagggctttgataagatgtactatgactacttccctgatgccgccaagatgatcccaaagtgcagcacccagctgaaggccgtgacagcccactttcagacccacacaacccccatcctgctgtccaacaatttcatcgagcctctggagatcacaaaggagatctacgacctgaacaatcctgagaaggagccaaagaagtttcagacagcctacgccaagaaaaccggcgaccagaagggctacagagaggccctgtgcaagtggatcgacttcacaagggattttctgtccaagtataccaagacaacctctatcgatctgtctagcctgcggccatcctctcagtataaggacctgggcgagtactatgccgagctgaatcccctgctgtaccacatcagcttccagagaatcgccgagaaggagatcatggatgccgtggagacaggcaagctgtacctgttccagatctataacaaggactttgccaagggccaccacggcaagcctaatctgcacacactgtattggaccggcctgttttctccagagaacctggccaagacaagcatcaagctgaatggccaggccgagctgttctaccgccctaagtccaggatgaagaggatggcacaccggctgggagagaagatgctgaacaagaagctgaaggatcagaaaaccccaatccccgacaccctgtaccaggagctgtacgactatgtgaatcacagactgtcccacgacctgtctgatgaggccagggccctgctgcccaacgtgatcaccaaggaggtgtctcacgagatcatcaaggataggcgctttaccagcgacaagttctttttccacgtgcctatcacactgaactatcaggccgccaattccccatctaagttcaaccagagggtgaatgcctacctgaaggagcaccccgagacacctatcatcggcatcgatcggggcgagagaaacctgatctatatcacagtgatcgactccaccggcaagatcctggagcagcggagcctgaacaccatccagcagtttgattaccagaagaagctggacaacagggagaaggagagggtggcagcaaggcaggcctggtctgtggtgggcacaatcaaggatctgaagcagggctatctgagccaggtcatccacgagatcgtggacctgatgatccactaccaggccgtggtggtgctggagaacctgaatttcggctttaagagcaagaggaccggcatcgccgagaaggccgtgtaccagcagttcgagaagatgctgatcgataagctgaattgcctggtgctgaaggactatccagcagagaaagtgggaggcgtgctgaacccataccagctgacagaccagttcacctcctttgccaagatgggcacccagtctggcttcctgttttacgtgcctgccccatatacatctaagatcgatcccctgaccggcttcgtggaccccttcgtgtggaaaaccatcaagaatcacgagagccgcaagcacttcctggagggcttcgactttctgcactacgacgtgaaaaccggcgacttcatcctgcactttaagatgaacagaaatctgtccttccagaggggcctgcccggctttatgcctgcatgggatatcgtgttcgagaagaacgagacacagtttgacgccaagggcacccctttcatcgccggcaagagaatcgtgccagtgatcgagaatcacagattcaccggcagataccgggacctgtatcctgccaacgagctgatcgccctgctggaggagaagggcatcgtgttcagggatggctccaacatcctgccaaagctgctggagaatgacgattctcacgccatcgacaccatggtggccctgatccgcagcgtgctgcagatgcggaactccaatgccgccacaggcgaggactatatcaacagccccgtgcgcgatctgaatggcgtgtgcttcgactcccggtttcagaacccagagtggcccatggacgccgatgccaatggcgcctaccacatcgccctgaagggccagctgctgctgaatcacctgaaggagagcaaggatctgaagctgcagaacggcatctccaatcaggactggctggcctacatccaggagctgcgcaac

SEQ ID NO: 64 - DNA, 189 bp, Artificial Sequence
  Exemplary DNA donor template containing only human KLF1 binding site
ttcatttttcattctcacaaactaatgaaaccctgcttatcttaaaccaacctgctcactggagcagggaggacaggaccagcataaaagccacaccctgcagggcagagtcgactgttgcttacactttcttctgacataacagtgttcactagcaacctcaaacagacaccatggtgcatctgactc

SEQ ID NO: 65 - DNA, 187 bp, Artificial Sequence
  DNA donor template containing only human b-DRF and TFIIB binding sites
ggaatagtggaatgaaggttcatttttcattctcacaaactaatgaaaccctgcttatcttaaaccaacctgctcactggagcagggagggcaggagccagggctgggcataaaaggcagggcagagtcgactgttgcttacactttcttctgacataacagtgttcactagcaacctcaaacagac

SEQ ID NO: 66 - DNA, 20 bp, Artificial Sequence
  qRT-PCR GAPDH forward primer
caacagcgacacccactcct

SEQ ID NO: 67 - DNA, 21 bp, Artificial Sequence
  qRT-PCR GAPDH reverse primer
caccctgttgctgtagccaaa

SEQ ID NO: 68 - DNA, 22 bp, Artificial Sequence
  qRT-PCR HBA forward primer
gaggccctggagaggatgttcc

SEQ ID NO: 69 - DNA, 22 bp, Artificial Sequence
  qRT-PCR HBA reverse primer
acagcgcgttgggcatgtcgtc

SEQ ID NO: 70 - DNA, 23 bp, Artificial Sequence
  qRT-PCR HBB forward primer
tgtccactcctgatgctgttatg

SEQ ID NO: 71 - DNA, 19 bp, Artificial Sequence
  qRT-PCR HBB reverse primer
ggcaccgagcactttcttg

SEQ ID NO: 72 - DNA, 21 bp, Artificial Sequence
  qRT-PCR HBD forward primer
aacctcaagggcactttttct

SEQ ID NO: 73 - DNA, 21 bp, Artificial Sequence
  qRT-PCR HBD reverse primer
ggaaacagtccaggatctcaa

SEQ ID NO: 74 - DNA, 19 bp, Artificial Sequence
  qRT-PCR HBG forward primer
cctgtcctctgcctctgcc

SEQ ID NO: 75 - DNA, 19 bp, Artificial Sequence
  qRT-PCR HBG reverse primer
ggattgccaaaacggtcac

SEQ ID NO: 76 - DNA, 28 bp, Artificial Sequence
  stubber sequence forward primer for NGS
ctttccctacacgacgctcttccgatct

SEQ ID NO: 77 - DNA, 28 bp, Artificial Sequence
  stubber sequence reverse primer for NGS
ggagttcagacgtgtgctcttccgatct

SEQ ID NO: 78 - DNA, 27 bp, Artificial Sequence
  NGS forward primer 1
cacacatgacagaacagccaatctcag

SEQ ID NO: 79 - DNA, 29 bp, Artificial Sequence
  NGS reverse primer 1
gaagaaagtgtaagcaacagtcgactctg

SEQ ID NO: 80 - DNA, 30 bp, Artificial Sequence
  NGS firward primer 2
gggcaagttaagggaatagtggaatgaagg

SEQ ID NO: 81 - DNA, 32 bp, Artificial Sequence
  NGS reverse primer 2
gaggttgctagtgaacactgttatgtcagaag

SEQ ID NO: 82 - DNA, 24 bp, Artificial Sequence
  ChIP-qPCR HBB forward primer
ccaactcctaagccagtgccagaa

SEQ ID NO: 83 - DNA, 27 bp, Artificial Sequence
  ChIP-qPCR HBB reverse primer
caaatgtaagcaatagatggctctgcc

SEQ ID NO: 84 - DNA, 30 bp, Artificial Sequence; identical to SEQ ID NO: 80
  ChIP-qPCR HBD forward primer

SEQ ID NO: 85 - DNA, 29 bp, Artificial Sequence
  ChIP-qPCR HBD reverse primer
gtcagaagaaagtgtaagcaacagtcgac

SEQ ID NO: 86 - DNA, 19 bp, Artificial Sequence
  ChIP-qPCR SP1 forward primer
acctctccgcccactagga

SEQ ID NO: 87 - DNA, 19 bp, Artificial Sequence
  ChIP-qPCR SP1 reverse primer
caacggccaaccagaatcc

SEQ ID NO: 88 - DNA, 20 bp, Artificial Sequence
  ChIP-qPCR AREG forward primer
tccacttcctctcagcgaat

SEQ ID NO: 89 - DNA, 20 bp, Artificial Sequence
  ChIP-qPCR AREG reverse primer
ggtgtgcgaacgtctgtagg

SEQ ID NO: 90 - DNA, 20 bp, Artificial Sequence
  ChIP-qPCR VEGFA forward primer
ggtttgtatcctgcccttcc

SEQ ID NO: 91 - DNA, 20 bp, Artificial Sequence
  ChIP-qPCR VEGFA reverse primer
actgggtcttgctgttttcc